European Patent Specification EP 4 027 144 B1, published February 12, 2025. Title: SYNTHETIC CONTROLS FOR IMMUNOHISTOCHEMISTRY. Applicant: Genentech, Inc. Hotzel, Kathy Peale Jr., Franklin V. Havnar, Charles Rangell, Linda Dunlap, Debra Y. Application Not Yet Assigned. The sequence listing filed with the application follows.

SEQUENCE LISTING (7 sequences)

SEQ ID NO: 1 - protein, 22 aa, Artificial Sequence
  Synthetic Construct
YGSGGAAPAPGIFSSQPGGSGC

SEQ ID NO: 2 - protein, 24 aa, Artificial Sequence
  Synthetic Construct
YGSGNRNYDLDYDSVQPYFYGSGC

SEQ ID NO: 3 - protein, 24 aa, Artificial Sequence
  Synthetic Construct
YGSGDSVQPYFYCDEEENFYGSGC

SEQ ID NO: 4 - protein, 24 aa, Artificial Sequence
  Synthetic Construct
YGSGQQQSELQPPAPSEDIWGSGC

SEQ ID NO: 5 - protein, 24 aa, Artificial Sequence
  Synthetic Construct
YGSGFELLPTPPLSPSRRSGGSGC

SEQ ID NO: 6 - protein, 4 aa, Artificial Sequence
  Synthetic Construct
YGSG

SEQ ID NO: 7 - protein, 4 aa, Artificial Sequence
  Synthetic Construct
GSGC